European Patent Specification EP 3 282 835 B1, published May 31, 2023. Title: GENETICALLY MODIFIED NON-HUMAN ANIMALS AND METHODS OF USE THEREOF. Applicant: Regeneron Pharmaceuticals, Inc. Herndler-Brandstetter, Dietmar Flavell, Richard Frleta, Davor Gurer, Cagan Manz, Markus Murphy, Andrew J. Palm, Noah W. Shan, Liang Stevens, Sean Strowig, Till Yancopoulos, George D. de Zoete, Marcel. The sequence listing filed with the application follows.

SEQUENCE LISTING (36 sequences)

SEQ ID NO: 1 - DNA, 200 bp, Artificial sequence
  synthetic polynucleotide
agctctcctaccactagactgctgagacccgctgctctgctcaggactcgatttccagtacacaatctccctctttgaaaagtaccacacatcctggggtgctcttgcatttgtgtgacactttgctagccaggctcagtcctgggttccaggtggggactcaaacacactggcacgagtctacattggatattcttggt

SEQ ID NO: 2 - DNA, 199 bp, Artificial sequence
  synthetic polynucleotide
gctccccattcctcactggcccagcccctcttccctactctttctagcccctgcctcatctccctggctgccattgggagcctgccccactggaagccagtcgagataacttcgtataatgtatgctatacgaagttatatgcatggcctccgcgccgggttttggcgcctcccgcgggcgcccccctcctcacggcga

SEQ ID NO: 3 - DNA, 200 bp, Artificial sequence
  synthetic polynucleotide
cattctcagtattgttttgccaagttctaattccatcagacctcgacctgcagcccctagataacttcgtataatgtatgctatacgaagttatgctagctgtctcatagaggctggcgatctggctcagggacagccagtactgcaaagagtatccttgttcataccttctcctagtggccatctccctgggacagtca

SEQ ID NO: 4 - DNA, 208 bp, Artificial sequence
  synthetic polynucleotide
atccatttagcctttctctgatcactaagttggacagttggacagtcttcctcaaattagcttagactatcaaaattatactgtatttttggtatttccagcgatcgcttcagttacaaggctgttgaatgcacagaagcaaggataacactgattttttcactggtcagaataaaaattattgattgctcttttgcttatagtattc

SEQ ID NO: 5 - DNA, 2028 bp, Artificial sequence
  synthetic polynucleotide
aatgtaacagaatctggatgcaaagaatgtgaggaactggaggaaaaaaatattaaagaatttttgcagagttttgtacatattgtccaaatgttcatcaacacttcttgattgcaattgattctttttaaagtgtttctgttattaacaaacatcactctgctgcttagacataacaaaacactcggcatttcaaatgtgctgtcaaaacaagtttttctgtcaagaagatgatcagaccttggatcagatgaactcttagaaatgaaggcagaaaaatgtcattgagtaatatagtgactatgaacttctctcagacttactttactcatttttttaatttattattgaaattgtacatatttgtggaataatgtaaaatgttgaataaaaatatgtacaagtgttgttttttaagttgcactgatattttacctcttattgcaaaatagcatttgtttaagggtgatagtcaaattatgtattggtggggctgggtaccaatgctgcaggtcaacagctatgctggtaggctcctgccagtgtggaaccactgactactggctctcattgacttccttactaagcatagcaaacagaggaagaatttgttatcagtaagaaaaagaagaactatatgtgaatcctcttctttatactgtaatttagttattgatgtataaagcaactgttatgaaataaagaaattgcaataactggcatataatgtccatcagtaaatcttggtggtggtggcaataataaacttctactgataggtagaatggtgtgcaagcttgtccaatcacggattgcaggccacatgcggcccaggacaactttgaatgtggcccaacacaaattcataaactttcatacatctcgtttttagctcatcagctatcattagcggtagtgtatttaaagtgtggcccaagacaattcttcttattccaatgtggcccagggaaatcaaaagattggatgcccctggtatagaaaactaatagtgacagtgttcatatttcatgctttcccaaatacaggtattttattttcacattctttttgccatgtttatataataataaagaaaaaccctgttgatttgttggagccattgttatctgacagaaaataattgtttatattttttgcactacactgtctaaaattagcaagctctcttctaatggaactgtaagaaagatgaaatatttttgttttattataaatttatttcaccttaattctggtaatactcactgagtgactgtggggtgggaaatgatctcttaagaatttgatttctttctattccatagtacaaactcgttctctgttgaaacattcttctatcaccccagtgccctatccatgtacatgtgttcttattgctctagtcaaacggtgcttataaatatctttcagaaagtttaggagaaatctgtatcctatttgacttccaataatcatgtattggctgtcagcttcttacctactctcagtccagagaaatagtatttggcagccactctttaaagtttatgggttgtggattgtggcggttgatttattttttttatttcaattgggatagaattttttaatatacctgtatttttgttttgttttatgtagcttttctattagggagagtaggaaaagtgcaccattttcttctctaaatttccagtccagtctttaggggaatgttagtcttcctgagatgggggaaggaaaatcataatgccagtcactttgcaaataatattttatagtgataaatggttcattttggttacataggcatacaagtgggcttaaaacttggaatttaccagggctcaaaattaaaattcttacattagttactcgatatggatcgcttcagttgatcttagaaaactcaaggcatagatctgcaacctcgagataacttcgtataatgtatgctatacgaagttatatgcatggcctccgcgccgggttttggcgcctcccgcgggcgcccccctcctcacggcg

SEQ ID NO: 6 - DNA, 200 bp, Artificial sequence
  synthetic polynucleotide
cattctcagtattgttttgccaagttctaattccatcagacctcgacctgcagcccctagataacttcgtataatgtatgctatacgaagttatgctagcgtgatagtccttcacggaaagtacaagaatacacagaaaactgctgtttacattagtctttcacgtttttattttattctcacaaattttaatgcaatac

SEQ ID NO: 7 - DNA, 20 bp, Artificial Sequence
  synthetic oligonucleotide
agggatttgaatcacgtttg

SEQ ID NO: 8 - DNA, 20 bp, Artificial Sequence
  synthetic oligonucleotide
tttactggcaacatcaacag

SEQ ID NO: 9 - DNA, 20 bp, Artificial Sequence
  synthetic oligonucleotide
gcccagggaaatcaaaagat

SEQ ID NO: 10 - DNA, 20 bp, Artificial Sequence
  synthetic oligonucleotide
tggctccaacaaatcaacag

SEQ ID NO: 11 - DNA, 4201 bp, Homo sapiens
tccggcccgcacccacccccaagaggggccttcagctttggggctcagaggcacgacctcctggggagggttaaaaggcagacgcccccccgccccccgcgcccccgcgccccgactccttcgccgcctccagcctctcgccagtgggaagcggggagcagccgcgcggccggagtccggaggcgaggggaggtcggccgcaacttccccggtccaccttaagaggacgatgtagccagctcgcagcgctgaccttagaaaaacaagtttgcgcaaagtggagcggggacccggcctctgggcagccccggcggcgcttccagtgccttccagccctcgcgggcggcgcagccgcggcccatggagcccgccggcccggcccccggccgcctcgggccgctgctctgcctgctgctcgccgcgtcctgcgcctggtcaggagtggcgggtgaggaggagctgcaggtgattcagcctgacaagtccgtgttggttgcagctggagagacagccactctgcgctgcactgcgacctctctgatccctgtggggcccatccagtggttcagaggagctggaccaggccgggaattaatctacaatcaaaaagaaggccacttcccccgggtaacaactgtttcagacctcacaaagagaaacaacatggacttttccatccgcatcggtaacatcaccccagcagatgccggcacctactactgtgtgaagttccggaaagggagccccgatgacgtggagtttaagtctggagcaggcactgagctgtctgtgcgcgccaaaccctctgcccccgtggtatcgggccctgcggcgagggccacacctcagcacacagtgagcttcacctgcgagtcccacggcttctcacccagagacatcaccctgaaatggttcaaaaatgggaatgagctctcagacttccagaccaacgtggaccccgtaggagagagcgtgtcctacagcatccacagcacagccaaggtggtgctgacccgcgaggacgttcactctcaagtcatctgcgaggtggcccacgtcaccttgcagggggaccctcttcgtgggactgccaacttgtctgagaccatccgagttccacccaccttggaggttactcaacagcccgtgagggcagagaaccaggtgaatgtcacctgccaggtgaggaagttctacccccagagactacagctgacctggttggagaatggaaacgtgtcccggacagaaacggcctcaaccgttacagagaacaaggatggtacctacaactggatgagctggctcctggtgaatgtatctgcccacagggatgatgtgaagctcacctgccaggtggagcatgacgggcagccagcggtcagcaaaagccatgacctgaaggtctcagcccacccgaaggagcagggctcaaataccgccgctgagaacactggatctaatgaacggaacatctatattgtggtgggtgtggtgtgcaccttgctggtggccctactgatggcggccctctacctcgtccgaatcagacagaagaaagcccagggctccacttcttctacaaggttgcatgagcccgagaagaatgccagagaaataacacaggacacaaatgatatcacatatgcagacctgaacctgcccaaggggaagaagcctgctccccaggctgcggagcccaacaaccacacggagtatgccagcattcagaccagcccgcagcccgcgtcggaggacaccctcacctatgctgacctggacatggtccacctcaaccggacccccaagcagccggcccccaagcctgagccgtccttctcagagtacgccagcgtccaggtcccgaggaagtgaatgggaccgtggtttgctctagcacccatctctacgcgctttcttgtcccacagggagccgccgtgatgagcacagccaacccagttcccggagggctggggcggtgcaggctctgggacccaggggccagggtggctcttctctccccacccctccttggctctccagcacttcctgggcagccacggccccctccccccacattgccacatacctggaggctgacgttgccaaaccagccagggaaccaacctgggaagtggccagaactgcctggggtccaagaactcttgtgcctccgtccatcaccatgtgggttttgaagaccctcgactgcctccccgatgctccgaagcctgatcttccagggtggggaggagaaaatcccacctcccctgacctccaccacctccaccaccaccaccaccaccaccaccaccactaccaccaccacccaactggggctagagtggggaagatttcccctttagatcaaactgccccttccatggaaaagctggaaaaaaactctggaacccatatccaggcttggtgaggttgctgccaacagtcctggcctcccccatccctaggctaaagagccatgagtcctggaggaggagaggacccctcccaaaggactggagacaaaaccctctgcttccttgggtccctccaagactccctggggcccaactgtgttgctccacccggacccatctctcccttctagacctgagcttgcccctccagctagcactaagcaacatctcgctgtggacgcctgtaaattactgagaaatgtgaaacgtgcaatcttgaaactgaggtgttagaaaacttgatctgtggtgttttgttttgttttttttcttaaaacaacagcaacgtgatcttggctgtctgtcatgtgttgaagtccatggttgggtcttgtgaagtctgaggtttaacagtttgttgtcctggagggattttcttacagcgaagacttgagttcctccaagtcccagaaccccaagaatgggcaagaaggatcaggtcagccactccctggagacacagccttctggctgggactgacttggccatgttctcagctgagccacgcggctggtagtgcagccttctgtgaccccgctgtggtaagtccagcctgcccagggctgctgagggctgcctcttgacagtgcagtcttatcgagacccaatgcctcagtctgctcatccgtaaagtggggatagtgaagatgacacccctccccaccacctctcataagcactttaggaacacacagagggtagggatagtggccctggccgtctatcctacccctttagtgaccgcccccatcccggctttctgagctgatccttgaagaagaaatcttccatttctgctctcaaaccctactgggatcaaactggaataaattgaagacagccagggggatggtgcagctgtgaagctcgggctgattccccctctgtcccagaaggttggccagagggtgtgacccagttaccctttaacccccacccttccagtcgggtgtgagggcctgaccgggcccagggcaagcagatgtcgcaagccctatttattcagtcttcactataactcttagagttgagacgctaatgttcatgactcctggccttgggatgcccaagggatttctggctcaggctgtaaaagtagctgagccatcctgcccattcctggaggtcctacaggtgaaactgcaggagctcagcatagacccagctctctgggggatggtcacctggtgatttcaatgatggcatccaggaattagctgagccaacagaccatgtggacagctttggccagagctcccgtgtggcatctgggagccacagtgacccagccacctggctcaggctagttccaaattccaaaagattggcttgtaaaccttcgtctccctctcttttacccagagacagcacatacgtgtgcacacgcatgcacacacacattcagtattttaaaagaatgttttcttggtgccattttcattttattttattttttaattcttggagggggaaataagggaataaggccaaggaagatgtatagctttagctttagcctggcaacctggagaatccacataccttgtgtattgaaccccaggaaaaggaagaggtcgaaccaaccctgcggaaggagcatggtttcaggagtttattttaagactgctgggaaggaaacaggccccattttgtatatagttgcaacttaaactttttggcttgcaaaatatttttgtaataaagatttctgggtaataatga

SEQ ID NO: 12 - protein, 504 aa, Homo sapiens
MEPAGPAPGRLGPLLCLLLAASCAWSGVAGEEELQVIQPDKSVLVAAGETATLRCTATSLIPVGPIQWFRGAGPGRELIYNQKEGHFPRVTTVSDLTKRNNMDFSIRIGNITPADAGTYYCVKFRKGSPDDVEFKSGAGTELSVRAKPSAPVVSGPAARATPQHTVSFTCESHGFSPRDITLKWFKNGNELSDFQTNVDPVGESVSYSIHSTAKVVLTREDVHSQVICEVAHVTLQGDPLRGTANLSETIRVPPTLEVTQQPVRAENQVNVTCQVRKFYPQRLQLTWLENGNVSRTETASTVTENKDGTYNWMSWLLVNVSAHRDDVKLTCQVEHDGQPAVSKSHDLKVSAHPKEQGSNTAAENTGSNERNIYIVVGVVCTLLVALLMAALYLVRIRQKKAQGSTSSTRLHEPEKNAREITQDTNDITYADLNLPKGKKPAPQAAEPNNHTEYASIQTSPQPASEDTLTYADLDMVHLNRTPKQPAPKPEPSFSEYASVQVPRK

SEQ ID NO: 13 - DNA, 4109 bp, Homo sapiens
ctctctggccgcccctggctttatttctcgcgcgcttggggtctctcccagtctccgtctctccatttctcctggggggcggggagggggggtctccaaaaaccgcggcggcggcggcggccgctccaggcgcccgttccggagtcggggggaggcccagccgggaggggggaagggggggagccttagtcatttccccgctccagcctgctcccgcccgagcgcgcactcacggccgctctccctcctcgctccgcagccgcggcccatggagcccgccggcccggcccccggccgcctcgggccgctgctctgcctgctgctcgccgcgtcctgcgcctggtcaggagtggcgggtgaggaggagctgcaggtgattcagcctgacaagtccgtgttggttgcagctggagagacagccactctgcgctgcactgcgacctctctgatccctgtggggcccatccagtggttcagaggagctggaccaggccgggaattaatctacaatcaaaaagaaggccacttcccccgggtaacaactgtttcagacctcacaaagagaaacaacatggacttttccatccgcatcggtaacatcaccccagcagatgccggcacctactactgtgtgaagttccggaaagggagccccgatgacgtggagtttaagtctggagcaggcactgagctgtctgtgcgcgccaaaccctctgcccccgtggtatcgggccctgcggcgagggccacacctcagcacacagtgagcttcacctgcgagtcccacggcttctcacccagagacatcaccctgaaatggttcaaaaatgggaatgagctctcagacttccagaccaacgtggaccccgtaggagagagcgtgtcctacagcatccacagcacagccaaggtggtgctgacccgcgaggacgttcactctcaagtcatctgcgaggtggcccacgtcaccttgcagggggaccctcttcgtgggactgccaacttgtctgagaccatccgagttccacccaccttggaggttactcaacagcccgtgagggcagagaaccaggtgaatgtcacctgccaggtgaggaagttctacccccagagactacagctgacctggttggagaatggaaacgtgtcccggacagaaacggcctcaaccgttacagagaacaaggatggtacctacaactggatgagctggctcctggtgaatgtatctgcccacagggatgatgtgaagctcacctgccaggtggagcatgacgggcagccagcggtcagcaaaagccatgacctgaaggtctcagcccacccgaaggagcagggctcaaataccgccgctgagaacactggatctaatgaacggaacatctatattgtggtgggtgtggtgtgcaccttgctggtggccctactgatggcggccctctacctcgtccgaatcagacagaagaaagcccagggctccacttcttctacaaggttgcatgagcccgagaagaatgccagagaaataacacaggacacaaatgatatcacatatgcagacctgaacctgcccaaggggaagaagcctgctccccaggctgcggagcccaacaaccacacggagtatgccagcattcagaccagcccgcagcccgcgtcggaggacaccctcacctatgctgacctggacatggtccacctcaaccggacccccaagcagccggcccccaagcctgagccgtccttctcagagtacgccagcgtccaggtcccgaggaagtgaatgggaccgtggtttgctctagcacccatctctacgcgctttcttgtcccacagggagccgccgtgatgagcacagccaacccagttcccggagggctggggcggtgcaggctctgggacccaggggccagggtggctcttctctccccacccctccttggctctccagcacttcctgggcagccacggccccctccccccacattgccacatacctggaggctgacgttgccaaaccagccagggaaccaacctgggaagtggccagaactgcctggggtccaagaactcttgtgcctccgtccatcaccatgtgggttttgaagaccctcgactgcctccccgatgctccgaagcctgatcttccagggtggggaggagaaaatcccacctcccctgacctccaccacctccaccaccaccaccaccaccaccaccaccactaccaccaccacccaactggggctagagtggggaagatttcccctttagatcaaactgccccttccatggaaaagctggaaaaaaactctggaacccatatccaggcttggtgaggttgctgccaacagtcctggcctcccccatccctaggctaaagagccatgagtcctggaggaggagaggacccctcccaaaggactggagacaaaaccctctgcttccttgggtccctccaagactccctggggcccaactgtgttgctccacccggacccatctctcccttctagacctgagcttgcccctccagctagcactaagcaacatctcgctgtggacgcctgtaaattactgagaaatgtgaaacgtgcaatcttgaaactgaggtgttagaaaacttgatctgtggtgttttgttttgttttttttcttaaaacaacagcaacgtgatcttggctgtctgtcatgtgttgaagtccatggttgggtcttgtgaagtctgaggtttaacagtttgttgtcctggagggattttcttacagcgaagacttgagttcctccaagtcccagaaccccaagaatgggcaagaaggatcaggtcagccactccctggagacacagccttctggctgggactgacttggccatgttctcagctgagccacgcggctggtagtgcagccttctgtgaccccgctgtggtaagtccagcctgcccagggctgctgagggctgcctcttgacagtgcagtcttatcgagacccaatgcctcagtctgctcatccgtaaagtggggatagtgaagatgacacccctccccaccacctctcataagcactttaggaacacacagagggtagggatagtggccctggccgtctatcctacccctttagtgaccgcccccatcccggctttctgagctgatccttgaagaagaaatcttccatttctgctctcaaaccctactgggatcaaactggaataaattgaagacagccagggggatggtgcagctgtgaagctcgggctgattccccctctgtcccagaaggttggccagagggtgtgacccagttaccctttaacccccacccttccagtcgggtgtgagggcctgaccgggcccagggcaagcagatgtcgcaagccctatttattcagtcttcactataactcttagagttgagacgctaatgttcatgactcctggccttgggatgcccaagggatttctggctcaggctgtaaaagtagctgagccatcctgcccattcctggaggtcctacaggtgaaactgcaggagctcagcatagacccagctctctgggggatggtcacctggtgatttcaatgatggcatccaggaattagctgagccaacagaccatgtggacagctttggccagagctcccgtgtggcatctgggagccacagtgacccagccacctggctcaggctagttccaaattccaaaagattggcttgtaaaccttcgtctccctctcttttacccagagacagcacatacgtgtgcacacgcatgcacacacacattcagtattttaaaagaatgttttcttggtgccattttcattttattttattttttaattcttggagggggaaataagggaataaggccaaggaagatgtatagctttagctttagcctggcaacctggagaatccacataccttgtgtattgaaccccaggaaaaggaagaggtcgaaccaaccctgcggaaggagcatggtttcaggagtttattttaagactgctgggaaggaaacaggccccattttgtatatagttgcaacttaaactttttggcttgcaaaatatttttgtaataaagatttctgggtaataatga

SEQ ID NO: 14 - DNA, 3868 bp, Homo sapiens
cgctcgctcgcagagaagccgcggcccatggagcccgccggcccggcccccggccgcctcgggccgctgctctgcctgctgctcgccgcgtcctgcgcctggtcaggagtggcgggtgaggaggagctgcaggtgattcagcctgacaagtccgtgttggttgcagctggagagacagccactctgcgctgcactgcgacctctctgatccctgtggggcccatccagtggttcagaggagctggaccaggccgggaattaatctacaatcaaaaagaaggccacttcccccgggtaacaactgtttcagacctcacaaagagaaacaacatggacttttccatccgcatcggtaacatcaccccagcagatgccggcacctactactgtgtgaagttccggaaagggagccccgatgacgtggagtttaagtctggagcaggcactgagctgtctgtgcgcgccaaaccctctgcccccgtggtatcgggccctgcggcgagggccacacctcagcacacagtgagcttcacctgcgagtcccacggcttctcacccagagacatcaccctgaaatggttcaaaaatgggaatgagctctcagacttccagaccaacgtggaccccgtaggagagagcgtgtcctacagcatccacagcacagccaaggtggtgctgacccgcgaggacgttcactctcaagtcatctgcgaggtggcccacgtcaccttgcagggggaccctcttcgtgggactgccaacttgtctgagaccatccgagttccacccaccttggaggttactcaacagcccgtgagggcagagaaccaggtgaatgtcacctgccaggtgaggaagttctacccccagagactacagctgacctggttggagaatggaaacgtgtcccggacagaaacggcctcaaccgttacagagaacaaggatggtacctacaactggatgagctggctcctggtgaatgtatctgcccacagggatgatgtgaagctcacctgccaggtggagcatgacgggcagccagcggtcagcaaaagccatgacctgaaggtctcagcccacccgaaggagcagggctcaaataccgccgctgagaacactggatctaatgaacggaacatctatattgtggtgggtgtggtgtgcaccttgctggtggccctactgatggcggccctctacctcgtccgaatcagacagaagaaagcccagggctccacttcttctacaaggttgcatgagcccgagaagaatgccagagaaataacacaggacacaaatgatatcacatatgcagacctgaacctgcccaaggggaagaagcctgctccccaggctgcggagcccaacaaccacacggagtatgccagcattcagaccagcccgcagcccgcgtcggaggacaccctcacctatgctgacctggacatggtccacctcaaccggacccccaagcagccggcccccaagcctgagccgtccttctcagagtacgccagcgtccaggtcccgaggaagtgaatgggaccgtggtttgctctagcacccatctctacgcgctttcttgtcccacagggagccgccgtgatgagcacagccaacccagttcccggagggctggggcggtgcaggctctgggacccaggggccagggtggctcttctctccccacccctccttggctctccagcacttcctgggcagccacggccccctccccccacattgccacatacctggaggctgacgttgccaaaccagccagggaaccaacctgggaagtggccagaactgcctggggtccaagaactcttgtgcctccgtccatcaccatgtgggttttgaagaccctcgactgcctccccgatgctccgaagcctgatcttccagggtggggaggagaaaatcccacctcccctgacctccaccacctccaccaccaccaccaccaccaccaccaccactaccaccaccacccaactggggctagagtggggaagatttcccctttagatcaaactgccccttccatggaaaagctggaaaaaaactctggaacccatatccaggcttggtgaggttgctgccaacagtcctggcctcccccatccctaggctaaagagccatgagtcctggaggaggagaggacccctcccaaaggactggagacaaaaccctctgcttccttgggtccctccaagactccctggggcccaactgtgttgctccacccggacccatctctcccttctagacctgagcttgcccctccagctagcactaagcaacatctcgctgtggacgcctgtaaattactgagaaatgtgaaacgtgcaatcttgaaactgaggtgttagaaaacttgatctgtggtgttttgttttgttttttttcttaaaacaacagcaacgtgatcttggctgtctgtcatgtgttgaagtccatggttgggtcttgtgaagtctgaggtttaacagtttgttgtcctggagggattttcttacagcgaagacttgagttcctccaagtcccagaaccccaagaatgggcaagaaggatcaggtcagccactccctggagacacagccttctggctgggactgacttggccatgttctcagctgagccacgcggctggtagtgcagccttctgtgaccccgctgtggtaagtccagcctgcccagggctgctgagggctgcctcttgacagtgcagtcttatcgagacccaatgcctcagtctgctcatccgtaaagtggggatagtgaagatgacacccctccccaccacctctcataagcactttaggaacacacagagggtagggatagtggccctggccgtctatcctacccctttagtgaccgcccccatcccggctttctgagctgatccttgaagaagaaatcttccatttctgctctcaaaccctactgggatcaaactggaataaattgaagacagccagggggatggtgcagctgtgaagctcgggctgattccccctctgtcccagaaggttggccagagggtgtgacccagttaccctttaacccccacccttccagtcgggtgtgagggcctgaccgggcccagggcaagcagatgtcgcaagccctatttattcagtcttcactataactcttagagttgagacgctaatgttcatgactcctggccttgggatgcccaagggatttctggctcaggctgtaaaagtagctgagccatcctgcccattcctggaggtcctacaggtgaaactgcaggagctcagcatagacccagctctctgggggatggtcacctggtgatttcaatgatggcatccaggaattagctgagccaacagaccatgtggacagctttggccagagctcccgtgtggcatctgggagccacagtgacccagccacctggctcaggctagttccaaattccaaaagattggcttgtaaaccttcgtctccctctcttttacccagagacagcacatacgtgtgcacacgcatgcacacacacattcagtattttaaaagaatgttttcttggtgccattttcattttattttattttttaattcttggagggggaaataagggaataaggccaaggaagatgtatagctttagctttagcctggcaacctggagaatccacataccttgtgtattgaaccccaggaaaaggaagaggtcgaaccaaccctgcggaaggagcatggtttcaggagtttattttaagactgctgggaaggaaacaggccccattttgtatatagttgcaacttaaactttttggcttgcaaaatatttttgtaataaagatttctgggtaataatga

SEQ ID NO: 15 - DNA, 4031 bp, Mus musculus
cgggaaggtgcgggcgcgaggagggggcgctcggccgggccgccctcgcgctggcctcgcgacggctccgcacagcccgcactcgctctgcgagctgtccccgctcgcgcttgctctccgatctccgtccccgctccctctccctcttcctctccccctctttccttctccctcgctatccgctcccccgcccccgtgcctctggctctgcgcctggctccctcgggtccgctcccctttcccgccggcctggcccggcgtcacgctcccggagtctccccgctcggcggcgtctcattgtgggagggggtcagatcaccccgccgggcggtggcgctggggggcagcggagggggaggggccttagtcgttcgcccgcgccgcccgcccgcctgccgagcgcgctcaccgccgctctccctccttgctctgcagccgcggcccatggagcccgccggcccggcccctggccgcctagggccgctgctgctctgcctgctgctctccgcgtcctgtttctgtacaggagccacggggaaggaactgaaggtgactcagcctgagaaatcagtgtctgttgctgctggggattcgaccgttctgaactgcactttgacctccttgttgccggtgggacccattaggtggtacagaggagtagggccaagccggctgttgatctacagtttcgcaggagaatacgttcctcgaattagaaatgtttcagatactactaagagaaacaatatggacttttccatccgtatcagtaatgtcaccccagcagatgctggcatctactactgtgtgaagttccagaaaggatcatcagagcctgacacagaaatacaatctggagggggaacagaggtctatgtactcgccaaaccttctccaccggaggtatccggcccagcagacaggggcatacctgaccagaaagtgaacttcacctgcaagtctcatggcttctctccccggaatatcaccctgaagtggttcaaagatgggcaagaactccaccccttggagaccaccgtgaaccctagtggaaagaatgtctcctacaacatctccagcacagtcagggtggtactaaactccatggatgttaattctaaggtcatctgcgaggtagcccacatcaccttggatagaagccctcttcgtgggattgctaacctgtctaacttcatccgagtttcacccaccgtgaaggtcacccaacagtccccgacgtcaatgaaccaggtgaacctcacctgccgggctgagaggttctaccccgaggatctccagctgatctggctggagaatggaaacgtatcacggaatgacacgcccaagaatctcacaaagaacacggatgggacctataattacacaagcttgttcctggtgaactcatctgctcatagagaggacgtggtgttcacgtgccaggtgaagcacgaccaacagccagcgatcacccgaaaccataccgtgctgggatttgcccactcgagtgatcaagggagcatgcaaaccttccctgataataatgctacccacaactggaatgtcttcatcggtgtgggcgtggcgtgtgctttgctcgtagtcctgctgatggctgctctctacctcctccggatcaaacagaagaaagccaaggggtcaacatcttccacacggttgcacgagcccgagaagaacgccagggaaataacccagatccaggacacaaatgacatcaacgacatcacatacgcagacctgaatctgcccaaagagaagaagcccgcaccccgggcccctgagcctaacaaccacacagaatatgcaagcattgagacaggcaaagtgcctaggccagaggataccctcacctatgctgacctggacatggtccacctcagccgggcacagccagcccccaagcctgagccatctttctcagagtatgctagtgtccaggtccagaggaagtgaatggggctgtggtctgtactaggccccatccccacaagttttcttgtcctacatggagtggccatgacgaggacatccagccagccaatcctgtccccagaaggccaggtggcacgggtcctaggaccaggggtaagggtggcctttgtcttccctccgtggctcttcaacacctcttgggcacccacgtccccttcttccggaggctgggtgttgcagaaccagagggcgaactggagaaagctgcctggaatccaagaagtgttgtgcctcggcccatcactcgtgggtctggatcctggtcttggcaaccccaggttgcgtccttgatgttccagagcttggtcttctgtgtggagaagagctcaccatctctacccaacttgagctttgggaccagactccctttagatcaaaccgccccatctgtggaagaactacaccagaagtcagcaagttttcagccaacagtgctggcctccccacctcccaggctgactagccctggggagaaggaaccctctcctcctagaccagcagagactccctgggcatgttcagtgtggccccacctcccttccagtcccagcttgcttcctccagctagcactaactcagcagcatcgctctgtggacgcctgtaaattattgagaaatgtgaactgtgcagtcttaaagctaaggtgttagaaaatttgatttatgctgtttagttgttgttgggtttcttttctttttaatttctttttcttttttgattttttttctttcccttaaaacaacagcagcagcatcttggctctttgtcatgtgttgaatggttgggtcttgtgaagtctgaggtctaacagtttattgtcctggaaggattttcttacagcagaaacagatttttttcaaattcccagaatcctgaggaccaagaaggatccctcagctgctacttccagcacccagcgtcactgggacgaaccaggccctgttcttacaaggccacatggctggccctttgcctccatggctactgtggtaagtgcagccttgtctgacccaatgctgacctaatgttggccattccacattgaggggacaaggtcagtgatgccccccttcactcacaagcacttcagaggcatgcagagagaagggacactcggccagctctctgaggtaatcagtgcaaggaggagtccgttttttgccagcaaacctcagcaggatcacactggaacagaacctggtcatacctgtgacaacacagctgtgagccagggcaaaccacccactgtcactggctcgagagtctgggcagaggctctgaccctccaccctttaaactggatgccggggcctggctgggcccaatgccaagtggttatggcaaccctgactatctggtcttaacatgtagctcaggaagtggaggcgctaatgtccccaatccctggggattcctgattccagctattcatgtaagcagagccaacctgcctatttctgtaggtgcgactgggatgttaggagcacagcaaggacccagctctgtagggctggtgacctgatacttctcataatggcatctagaagttaggctgagttggcctcactggcccagcaaaccagaacttgtctttgtccgggccatgttcttgggctgtcttctaattccaaagggttggttggtaaagctccacccccttctcctctgcctaaagacatcacatgtgtatacacacacgggtgtatagatgagttaaaagaatgtcctcgctggcatcctaattttgtcttaagtttttttggagggagaaaggaacaaggcaagggaagatgtgtagctttggctttaaccaggcagcctgggggctcccaagcctatggaaccctggtacaaagaagagaacagaagcgccctgtgaggagtgggatttgtttttctgtagaccagatgagaaggaaacaggccctgttttgtacatagttgcaacttaaaatttttggcttgcaaaatatttttgtaataaagatttctgggtaacaataaaaaaaaaaaaaaa

SEQ ID NO: 16 - protein, 509 aa, Mus musculus
MEPAGPAPGRLGPLLLCLLLSASCFCTGATGKELKVTQPEKSVSVAAGDSTVLNCTLTSLLPVGPIRWYRGVGPSRLLIYSFAGEYVPRIRNVSDTTKRNNMDFSIRISNVTPADAGIYYCVKFQKGSSEPDTEIQSGGGTEVYVLAKPSPPEVSGPADRGIPDQKVNFTCKSHGFSPRNITLKWFKDGQELHPLETTVNPSGKNVSYNISSTVRVVLNSMDVNSKVICEVAHITLDRSPLRGIANLSNFIRVSPTVKVTQQSPTSMNQVNLTCRAERFYPEDLQLIWLENGNVSRNDTPKNLTKNTDGTYNYTSLFLVNSSAHREDVVFTCQVKHDQQPAITRNHTVLGFAHSSDQGSMQTFPDNNATHNWNVFIGVGVACALLVVLLMAALYLLRIKQKKAKGSTSSTRLHEPEKNAREITQIQDTNDINDITYADLNLPKEKKPAPRAPEPNNHTEYASIETGKVPRPEDTLTYADLDMVHLSRAQPAPKPEPSFSEYASVQVQRK

SEQ ID NO: 17 - DNA, 3377 bp, Mus musculus
cgggaaggtgcgggcgcgaggagggggcgctcggccgggccgccctcgcgctggcctcgcgacggctccgcacagcccgcactcgctctgcgagctgtccccgctcgcgcttgctctccgatctccgtccccgctccctctccctcttcctctccccctctttccttctccctcgctatccgctcccccgcccccgtgcctctggctctgcgcctggctccctcgggtccgctcccctttcccgccggcctggcccggcgtcacgctcccggagtctccccgctcggcggcgtctcattgtgggagggggtcagatcaccccgccgggcggtggcgctggggggcagcggagggggaggggccttagtcgttcgcccgcgccgcccgcccgcctgccgagcgcgctcaccgccgctctccctccttgctctgcagccgcggcccatggagcccgccggcccggcccctggccgcctagggccgctgctgctctgcctgctgctctccgcgtcctgtttctgtacaggagccacggggaaggaactgaaggtgactcagcctgagaaatcagtgtctgttgctgctggggattcgaccgttctgaactgcactttgacctccttgttgccggtgggacccattaggtggtacagaggagtagggccaagccggctgttgatctacagtttcgcaggagaatacgttcctcgaattagaaatgtttcagatactactaagagaaacaatatggacttttccatccgtatcagtaatgtcaccccagcagatgctggcatctactactgtgtgaagttccagaaaggatcatcagagcctgacacagaaatacaatctggagggggaacagaggtctatgtactcgataataatgctacccacaactggaatgtcttcatcggtgtgggcgtggcgtgtgctttgctcgtagtcctgctgatggctgctctctacctcctccggatcaaacagaagaaagccaaggggtcaacatcttccacacggttgcacgagcccgagaagaacgccagggaaataacccagatccaggacacaaatgacatcaacgacatcacatacgcagacctgaatctgcccaaagagaagaagcccgcaccccgggcccctgagcctaacaaccacacagaatatgcaagcattgagacaggcaaagtgcctaggccagaggataccctcacctatgctgacctggacatggtccacctcagccgggcacagccagcccccaagcctgagccatctttctcagagtatgctagtgtccaggtccagaggaagtgaatggggctgtggtctgtactaggccccatccccacaagttttcttgtcctacatggagtggccatgacgaggacatccagccagccaatcctgtccccagaaggccaggtggcacgggtcctaggaccaggggtaagggtggcctttgtcttccctccgtggctcttcaacacctcttgggcacccacgtccccttcttccggaggctgggtgttgcagaaccagagggcgaactggagaaagctgcctggaatccaagaagtgttgtgcctcggcccatcactcgtgggtctggatcctggtcttggcaaccccaggttgcgtccttgatgttccagagcttggtcttctgtgtggagaagagctcaccatctctacccaacttgagctttgggaccagactccctttagatcaaaccgccccatctgtggaagaactacaccagaagtcagcaagttttcagccaacagtgctggcctccccacctcccaggctgactagccctggggagaaggaaccctctcctcctagaccagcagagactccctgggcatgttcagtgtggccccacctcccttccagtcccagcttgcttcctccagctagcactaactcagcagcatcgctctgtggacgcctgtaaattattgagaaatgtgaactgtgcagtcttaaagctaaggtgttagaaaatttgatttatgctgtttagttgttgttgggtttcttttctttttaatttctttttcttttttgattttttttctttcccttaaaacaacagcagcagcatcttggctctttgtcatgtgttgaatggttgggtcttgtgaagtctgaggtctaacagtttattgtcctggaaggattttcttacagcagaaacagatttttttcaaattcccagaatcctgaggaccaagaaggatccctcagctgctacttccagcacccagcgtcactgggacgaaccaggccctgttcttacaaggccacatggctggccctttgcctccatggctactgtggtaagtgcagccttgtctgacccaatgctgacctaatgttggccattccacattgaggggacaaggtcagtgatgccccccttcactcacaagcacttcagaggcatgcagagagaagggacactcggccagctctctgaggtaatcagtgcaaggaggagtccgttttttgccagcaaacctcagcaggatcacactggaacagaacctggtcatacctgtgacaacacagctgtgagccagggcaaaccacccactgtcactggctcgagagtctgggcagaggctctgaccctccaccctttaaactggatgccggggcctggctgggcccaatgccaagtggttatggcaaccctgactatctggtcttaacatgtagctcaggaagtggaggcgctaatgtccccaatccctggggattcctgattccagctattcatgtaagcagagccaacctgcctatttctgtaggtgcgactgggatgttaggagcacagcaaggacccagctctgtagggctggtgacctgatacttctcataatggcatctagaagttaggctgagttggcctcactggcccagcaaaccagaacttgtctttgtccgggccatgttcttgggctgtcttctaattccaaagggttggttggtaaagctccacccccttctcctctgcctaaagacatcacatgtgtatacacacacgggtgtatagatgagttaaaagaatgtcctcgctggcatcctaattttgtcttaagtttttttggagggagaaaggaacaaggcaagggaagatgtgtagctttggctttaaccaggcagcctgggggctcccaagcctatggaaccctggtacaaagaagagaacagaagcgccctgtgaggagtgggatttgtttttctgtagaccagatgagaaggaaacaggccctgttttgtacatagttgcaacttaaaatttttggcttgcaaaatatttttgtaataaagatttctgggtaacaataaaaaaaaaaaaaaa

SEQ ID NO: 18 - protein, 291 aa, Mus musculus
MEPAGPAPGRLGPLLLCLLLSASCFCTGATGKELKVTQPEKSVSVAAGDSTVLNCTLTSLLPVGPIRWYRGVGPSRLLIYSFAGEYVPRIRNVSDTTKRNNMDFSIRISNVTPADAGIYYCVKFQKGSSEPDTEIQSGGGTEVYVLDNNATHNWNVFIGVGVACALLVVLLMAALYLLRIKQKKAKGSTSSTRLHEPEKNAREITQIQDTNDINDITYADLNLPKEKKPAPRAPEPNNHTEYASIETGKVPRPEDTLTYADLDMVHLSRAQPAPKPEPSFSEYASVQVQRK

SEQ ID NO: 19 - DNA, 4043 bp, Mus musculus
cgggaaggtgcgggcgcgaggagggggcgctcggccgggccgccctcgcgctggcctcgcgacggctccgcacagcccgcactcgctctgcgagctgtccccgctcgcgcttgctctccgatctccgtccccgctccctctccctcttcctctccccctctttccttctccctcgctatccgctcccccgcccccgtgcctctggctctgcgcctggctccctcgggtccgctcccctttcccgccggcctggcccggcgtcacgctcccggagtctccccgctcggcggcgtctcattgtgggagggggtcagatcaccccgccgggcggtggcgctggggggcagcggagggggaggggccttagtcgttcgcccgcgccgcccgcccgcctgccgagcgcgctcaccgccgctctccctccttgctctgcagccgcggcccatggagcccgccggcccggcccctggccgcctagggccgctgctgctctgcctgctgctctccgcgtcctgtttctgtacaggagccacggggaaggaactgaaggtgactcagcctgagaaatcagtgtctgttgctgctggggattcgaccgttctgaactgcactttgacctccttgttgccggtgggacccattaggtggtacagaggagtagggccaagccggctgttgatctacagtttcgcaggagaatacgttcctcgaattagaaatgtttcagatactactaagagaaacaatatggacttttccatccgtatcagtaatgtcaccccagcagatgctggcatctactactgtgtgaagttccagaaaggatcatcagagcctgacacagaaatacaatctggagggggaacagaggtctatgtactcgccaaaccttctccaccggaggtatccggcccagcagacaggggcatacctgaccagaaagtgaacttcacctgcaagtctcatggcttctctccccggaatatcaccctgaagtggttcaaagatgggcaagaactccaccccttggagaccaccgtgaaccctagtggaaagaatgtctcctacaacatctccagcacagtcagggtggtactaaactccatggatgttaattctaaggtcatctgcgaggtagcccacatcaccttggatagaagccctcttcgtgggattgctaacctgtctaacttcatccgagtttcacccaccgtgaaggtcacccaacagtccccgacgtcaatgaaccaggtgaacctcacctgccgggctgagaggttctaccccgaggatctccagctgatctggctggagaatggaaacgtatcacggaatgacacgcccaagaatctcacaaagaacacggatgggacctataattacacaagcttgttcctggtgaactcatctgctcatagagaggacgtggtgttcacgtgccaggtgaagcacgaccaacagccagcgatcacccgaaaccataccgtgctgggatttgcccactcgagtgatcaagggagcatgcaaaccttccctgataataatgctacccacaactggaatgtcttcatcggtgtgggcgtggcgtgtgctttgctcgtagtcctgctgatggctgctctctacctcctccggatcaaacagaagaaagccaaggggtcaacatcttccacacggttgcacgagcccgagaagaacgccagggaaataacccaggtacagtctttgatccaggacacaaatgacatcaacgacatcacatacgcagacctgaatctgcccaaagagaagaagcccgcaccccgggcccctgagcctaacaaccacacagaatatgcaagcattgagacaggcaaagtgcctaggccagaggataccctcacctatgctgacctggacatggtccacctcagccgggcacagccagcccccaagcctgagccatctttctcagagtatgctagtgtccaggtccagaggaagtgaatggggctgtggtctgtactaggccccatccccacaagttttcttgtcctacatggagtggccatgacgaggacatccagccagccaatcctgtccccagaaggccaggtggcacgggtcctaggaccaggggtaagggtggcctttgtcttccctccgtggctcttcaacacctcttgggcacccacgtccccttcttccggaggctgggtgttgcagaaccagagggcgaactggagaaagctgcctggaatccaagaagtgttgtgcctcggcccatcactcgtgggtctggatcctggtcttggcaaccccaggttgcgtccttgatgttccagagcttggtcttctgtgtggagaagagctcaccatctctacccaacttgagctttgggaccagactccctttagatcaaaccgccccatctgtggaagaactacaccagaagtcagcaagttttcagccaacagtgctggcctccccacctcccaggctgactagccctggggagaaggaaccctctcctcctagaccagcagagactccctgggcatgttcagtgtggccccacctcccttccagtcccagcttgcttcctccagctagcactaactcagcagcatcgctctgtggacgcctgtaaattattgagaaatgtgaactgtgcagtcttaaagctaaggtgttagaaaatttgatttatgctgtttagttgttgttgggtttcttttctttttaatttctttttcttttttgattttttttctttcccttaaaacaacagcagcagcatcttggctctttgtcatgtgttgaatggttgggtcttgtgaagtctgaggtctaacagtttattgtcctggaaggattttcttacagcagaaacagatttttttcaaattcccagaatcctgaggaccaagaaggatccctcagctgctacttccagcacccagcgtcactgggacgaaccaggccctgttcttacaaggccacatggctggccctttgcctccatggctactgtggtaagtgcagccttgtctgacccaatgctgacctaatgttggccattccacattgaggggacaaggtcagtgatgccccccttcactcacaagcacttcagaggcatgcagagagaagggacactcggccagctctctgaggtaatcagtgcaaggaggagtccgttttttgccagcaaacctcagcaggatcacactggaacagaacctggtcatacctgtgacaacacagctgtgagccagggcaaaccacccactgtcactggctcgagagtctgggcagaggctctgaccctccaccctttaaactggatgccggggcctggctgggcccaatgccaagtggttatggcaaccctgactatctggtcttaacatgtagctcaggaagtggaggcgctaatgtccccaatccctggggattcctgattccagctattcatgtaagcagagccaacctgcctatttctgtaggtgcgactgggatgttaggagcacagcaaggacccagctctgtagggctggtgacctgatacttctcataatggcatctagaagttaggctgagttggcctcactggcccagcaaaccagaacttgtctttgtccgggccatgttcttgggctgtcttctaattccaaagggttggttggtaaagctccacccccttctcctctgcctaaagacatcacatgtgtatacacacacgggtgtatagatgagttaaaagaatgtcctcgctggcatcctaattttgtcttaagtttttttggagggagaaaggaacaaggcaagggaagatgtgtagctttggctttaaccaggcagcctgggggctcccaagcctatggaaccctggtacaaagaagagaacagaagcgccctgtgaggagtgggatttgtttttctgtagaccagatgagaaggaaacaggccctgttttgtacatagttgcaacttaaaatttttggcttgcaaaatatttttgtaataaagatttctgggtaacaataaaaaaaaaaaaaaa

SEQ ID NO: 20 - protein, 513 aa, Mus musculus
MEPAGPAPGRLGPLLLCLLLSASCFCTGATGKELKVTQPEKSVSVAAGDSTVLNCTLTSLLPVGPIRWYRGVGPSRLLIYSFAGEYVPRIRNVSDTTKRNNMDFSIRISNVTPADAGIYYCVKFQKGSSEPDTEIQSGGGTEVYVLAKPSPPEVSGPADRGIPDQKVNFTCKSHGFSPRNITLKWFKDGQELHPLETTVNPSGKNVSYNISSTVRVVLNSMDVNSKVICEVAHITLDRSPLRGIANLSNFIRVSPTVKVTQQSPTSMNQVNLTCRAERFYPEDLQLIWLENGNVSRNDTPKNLTKNTDGTYNYTSLFLVNSSAHREDVVFTCQVKHDQQPAITRNHTVLGFAHSSDQGSMQTFPDNNATHNWNVFIGVGVACALLVVLLMAALYLLRIKQKKAKGSTSSTRLHEPEKNAREITQVQSLIQDTNDINDITYADLNLPKEKKPAPRAPEPNNHTEYASIETGKVPRPEDTLTYADLDMVHLSRAQPAPKPEPSFSEYASVQVQRK

SEQ ID NO: 21 - DNA, 3845 bp, Mus musculus
aagctcccctgccgcgggcagcctcttgcccactggagtctaaggactggccgggtgagaggccgagaccagggggcgatcggccgccacttccccagtccaccttaagaggaccaagtagccagcccgccgcgccgacctcagaaaaacaagtttgcgcaaagtggtgcgcggccagcctctgggcagagggagcggtgcttccaccgcctggcagccctgcgcgcggcggcgcagccgcggcccatggagcccgccggcccggcccctggccgcctagggccgctgctgctctgcctgctgctctccgcgtcctgtttctgtacaggagccacggggaaggaactgaaggtgactcagcctgagaaatcagtgtctgttgctgctggggattcgaccgttctgaactgcactttgacctccttgttgccggtgggacccattaggtggtacagaggagtagggccaagccggctgttgatctacagtttcgcaggagaatacgttcctcgaattagaaatgtttcagatactactaagagaaacaatatggacttttccatccgtatcagtaatgtcaccccagcagatgctggcatctactactgtgtgaagttccagaaaggatcatcagagcctgacacagaaatacaatctggagggggaacagaggtctatgtactcgccaaaccttctccaccggaggtatccggcccagcagacaggggcatacctgaccagaaagtgaacttcacctgcaagtctcatggcttctctccccggaatatcaccctgaagtggttcaaagatgggcaagaactccaccccttggagaccaccgtgaaccctagtggaaagaatgtctcctacaacatctccagcacagtcagggtggtactaaactccatggatgttaattctaaggtcatctgcgaggtagcccacatcaccttggatagaagccctcttcgtgggattgctaacctgtctaacttcatccgagtttcacccaccgtgaaggtcacccaacagtccccgacgtcaatgaaccaggtgaacctcacctgccgggctgagaggttctaccccgaggatctccagctgatctggctggagaatggaaacgtatcacggaatgacacgcccaagaatctcacaaagaacacggatgggacctataattacacaagcttgttcctggtgaactcatctgctcatagagaggacgtggtgttcacgtgccaggtgaagcacgaccaacagccagcgatcacccgaaaccataccgtgctgggatttgcccactcgagtgatcaagggagcatgcaaaccttccctgataataatgctacccacaactggaatgtcttcatcggtgtgggcgtggcgtgtgctttgctcgtagtcctgctgatggctgctctctacctcctccggatcaaacagaagaaagccaaggggtcaacatcttccacacggttgcacgagcccgagaagaacgccagggaaataacccaggtacagtctttgatccaggacacaaatgacatcaacgacatcacatacgcagacctgaatctgcccaaagagaagaagcccgcaccccgggcccctgagcctaacaaccacacagaatatgcaagcattgagacaggcaaagtgcctaggccagaggataccctcacctatgctgacctggacatggtccacctcagccgggcacagccagcccccaagcctgagccatctttctcagagtatgctagtgtccaggtccagaggaagtgaatggggctgtggtctgtactaggccccatccccacaagttttcttgtcctacatggagtggccatgacgaggacatccagccagccaatcctgtccccagaaggccaggtggcacgggtcctaggaccaggggtaagggtggcctttgtcttccctccgtggctcttcaacacctcttgggcacccacgtccccttcttccggaggctgggtgttgcagaaccagagggcgaactggagaaagctgcctggaatccaagaagtgttgtgcctcggcccatcactcgtgggtctggatcctggtcttggcaaccccaggttgcgtccttgatgttccagagcttggtcttctgtgtggagaagagctcaccatctctacccaacttgagctttgggaccagactccctttagatcaaaccgccccatctgtggaagaactacaccagaagtcagcaagttttcagccaacagtgctggcctccccacctcccaggctgactagccctggggagaaggaaccctctcctcctagaccagcagagactccctgggcatgttcagtgtggccccacctcccttccagtcccagcttgcttcctccagctagcactaactcagcagcatcgctctgtggacgcctgtaaattattgagaaatgtgaactgtgcagtcttaaagctaaggtgttagaaaatttgatttatgctgtttagttgttgttgggtttcttttctttttaatttctttttcttttttgattttttttctttcccttaaaacaacagcagcagcatcttggctctttgtcatgtgttgaatggttgggtcttgtgaagtctgaggtctaacagtttattgtcctggaaggattttcttacagcagaaacagatttttttcaaattcccagaatcctgaggaccaagaaggatccctcagctgctacttccagcacccagcgtcactgggacgaaccaggccctgttcttacaaggccacatggctggccctttgcctccatggctactgtggtaagtgcagccttgtctgacccaatgctgacctaatgttggccattccacattgaggggacaaggtcagtgatgccccccttcactcacaagcacttcagaggcatgcagagagaagggacactcggccagctctctgaggtaatcagtgcaaggaggagtccgttttttgccagcaaacctcagcaggatcacactggaacagaacctggtcatacctgtgacaacacagctgtgagccagggcaaaccacccactgtcactggctcgagagtctgggcagaggctctgaccctccaccctttaaactggatgccggggcctggctgggcccaatgccaagtggttatggcaaccctgactatctggtcttaacatgtagctcaggaagtggaggcgctaatgtccccaatccctggggattcctgattccagctattcatgtaagcagagccaacctgcctatttctgtaggtgcgactgggatgttaggagcacagcaaggacccagctctgtagggctggtgacctgatacttctcataatggcatctagaagttaggctgagttggcctcactggcccagcaaaccagaacttgtctttgtccgggccatgttcttgggctgtcttctaattccaaagggttggttggtaaagctccacccccttctcctctgcctaaagacatcacatgtgtatacacacacgggtgtatagatgagttaaaagaatgtcctcgctggcatcctaattttgtcttaagtttttttggagggagaaaggaacaaggcaagggaagatgtgtagctttggctttaaccaggcagcctgggggctcccaagcctatggaaccctggtacaaagaagagaacagaagcgccctgtgaggagtgggatttgtttttctgtagaccagatgagaaggaaacaggccctgttttgtacatagttgcaacttaaaatttttggcttgcaaaatatttttgtaataaagatttctgggtaacaataaaaaaaaaaaaaaa

SEQ ID NO: 22 - DNA, 3389 bp, Mus musculus
cgggaaggtgcgggcgcgaggagggggcgctcggccgggccgccctcgcgctggcctcgcgacggctccgcacagcccgcactcgctctgcgagctgtccccgctcgcgcttgctctccgatctccgtccccgctccctctccctcttcctctccccctctttccttctccctcgctatccgctcccccgcccccgtgcctctggctctgcgcctggctccctcgggtccgctcccctttcccgccggcctggcccggcgtcacgctcccggagtctccccgctcggcggcgtctcattgtgggagggggtcagatcaccccgccgggcggtggcgctggggggcagcggagggggaggggccttagtcgttcgcccgcgccgcccgcccgcctgccgagcgcgctcaccgccgctctccctccttgctctgcagccgcggcccatggagcccgccggcccggcccctggccgcctagggccgctgctgctctgcctgctgctctccgcgtcctgtttctgtacaggagccacggggaaggaactgaaggtgactcagcctgagaaatcagtgtctgttgctgctggggattcgaccgttctgaactgcactttgacctccttgttgccggtgggacccattaggtggtacagaggagtagggccaagccggctgttgatctacagtttcgcaggagaatacgttcctcgaattagaaatgtttcagatactactaagagaaacaatatggacttttccatccgtatcagtaatgtcaccccagcagatgctggcatctactactgtgtgaagttccagaaaggatcatcagagcctgacacagaaatacaatctggagggggaacagaggtctatgtactcgataataatgctacccacaactggaatgtcttcatcggtgtgggcgtggcgtgtgctttgctcgtagtcctgctgatggctgctctctacctcctccggatcaaacagaagaaagccaaggggtcaacatcttccacacggttgcacgagcccgagaagaacgccagggaaataacccaggtacagtctttgatccaggacacaaatgacatcaacgacatcacatacgcagacctgaatctgcccaaagagaagaagcccgcaccccgggcccctgagcctaacaaccacacagaatatgcaagcattgagacaggcaaagtgcctaggccagaggataccctcacctatgctgacctggacatggtccacctcagccgggcacagccagcccccaagcctgagccatctttctcagagtatgctagtgtccaggtccagaggaagtgaatggggctgtggtctgtactaggccccatccccacaagttttcttgtcctacatggagtggccatgacgaggacatccagccagccaatcctgtccccagaaggccaggtggcacgggtcctaggaccaggggtaagggtggcctttgtcttccctccgtggctcttcaacacctcttgggcacccacgtccccttcttccggaggctgggtgttgcagaaccagagggcgaactggagaaagctgcctggaatccaagaagtgttgtgcctcggcccatcactcgtgggtctggatcctggtcttggcaaccccaggttgcgtccttgatgttccagagcttggtcttctgtgtggagaagagctcaccatctctacccaacttgagctttgggaccagactccctttagatcaaaccgccccatctgtggaagaactacaccagaagtcagcaagttttcagccaacagtgctggcctccccacctcccaggctgactagccctggggagaaggaaccctctcctcctagaccagcagagactccctgggcatgttcagtgtggccccacctcccttccagtcccagcttgcttcctccagctagcactaactcagcagcatcgctctgtggacgcctgtaaattattgagaaatgtgaactgtgcagtcttaaagctaaggtgttagaaaatttgatttatgctgtttagttgttgttgggtttcttttctttttaatttctttttcttttttgattttttttctttcccttaaaacaacagcagcagcatcttggctctttgtcatgtgttgaatggttgggtcttgtgaagtctgaggtctaacagtttattgtcctggaaggattttcttacagcagaaacagatttttttcaaattcccagaatcctgaggaccaagaaggatccctcagctgctacttccagcacccagcgtcactgggacgaaccaggccctgttcttacaaggccacatggctggccctttgcctccatggctactgtggtaagtgcagccttgtctgacccaatgctgacctaatgttggccattccacattgaggggacaaggtcagtgatgccccccttcactcacaagcacttcagaggcatgcagagagaagggacactcggccagctctctgaggtaatcagtgcaaggaggagtccgttttttgccagcaaacctcagcaggatcacactggaacagaacctggtcatacctgtgacaacacagctgtgagccagggcaaaccacccactgtcactggctcgagagtctgggcagaggctctgaccctccaccctttaaactggatgccggggcctggctgggcccaatgccaagtggttatggcaaccctgactatctggtcttaacatgtagctcaggaagtggaggcgctaatgtccccaatccctggggattcctgattccagctattcatgtaagcagagccaacctgcctatttctgtaggtgcgactgggatgttaggagcacagcaaggacccagctctgtagggctggtgacctgatacttctcataatggcatctagaagttaggctgagttggcctcactggcccagcaaaccagaacttgtctttgtccgggccatgttcttgggctgtcttctaattccaaagggttggttggtaaagctccacccccttctcctctgcctaaagacatcacatgtgtatacacacacgggtgtatagatgagttaaaagaatgtcctcgctggcatcctaattttgtcttaagtttttttggagggagaaaggaacaaggcaagggaagatgtgtagctttggctttaaccaggcagcctgggggctcccaagcctatggaaccctggtacaaagaagagaacagaagcgccctgtgaggagtgggatttgtttttctgtagaccagatgagaaggaaacaggccctgttttgtacatagttgcaacttaaaatttttggcttgcaaaatatttttgtaataaagatttctgggtaacaataaaaaaaaaaaaaaa

SEQ ID NO: 23 - protein, 295 aa, Mus musculus
MEPAGPAPGRLGPLLLCLLLSASCFCTGATGKELKVTQPEKSVSVAAGDSTVLNCTLTSLLPVGPIRWYRGVGPSRLLIYSFAGEYVPRIRNVSDTTKRNNMDFSIRISNVTPADAGIYYCVKFQKGSSEPDTEIQSGGGTEVYVLDNNATHNWNVFIGVGVACALLVVLLMAALYLLRIKQKKAKGSTSSTRLHEPEKNAREITQVQSLIQDTNDINDITYADLNLPKEKKPAPRAPEPNNHTEYASIETGKVPRPEDTLTYADLDMVHLSRAQPAPKPEPSFSEYASVQVQRK

SEQ ID NO: 24 - DNA, 3020 bp, Mus musculus
cgggaaggtgcgggcgcgaggagggggcgctcggccgggccgccctcgcgctggcctcgcgacggctccgcacagcccgcactcgctctgcgagctgtccccgctcgcgcttgctctccgatctccgtccccgctccctctccctcttcctctccccctctttccttctccctcgctatccgctcccccgcccccgtgcctctggctctgcgcctggctccctcgggtccgctcccctttcccgccggcctggcccggcgtcacgctcccggagtctccccgctcggcggcgtctcattgtgggagggggtcagatcaccccgccgggcggtggcgctggggggcagcggagggggaggggccttagtcgttcgcccgcgccgcccgcccgcctgccgagcgcgctcaccgccgctctccctccttgctctgcagccgcggcccatggagcccgccggcccggcccctggccgcctagggccgctgctgctctgcctgctgctctccgcgtcctgtttctgtacagataataatgctacccacaactggaatgtcttcatcggtgtgggcgtggcgtgtgctttgctcgtagtcctgctgatggctgctctctacctcctccggatcaaacagaagaaagccaaggggtcaacatcttccacacggttgcacgagcccgagaagaacgccagggaaataacccagatccaggacacaaatgacatcaacgacatcacatacgcagacctgaatctgcccaaagagaagaagcccgcaccccgggcccctgagcctaacaaccacacagaatatgcaagcattgagacaggcaaagtgcctaggccagaggataccctcacctatgctgacctggacatggtccacctcagccgggcacagccagcccccaagcctgagccatctttctcagagtatgctagtgtccaggtccagaggaagtgaatggggctgtggtctgtactaggccccatccccacaagttttcttgtcctacatggagtggccatgacgaggacatccagccagccaatcctgtccccagaaggccaggtggcacgggtcctaggaccaggggtaagggtggcctttgtcttccctccgtggctcttcaacacctcttgggcacccacgtccccttcttccggaggctgggtgttgcagaaccagagggcgaactggagaaagctgcctggaatccaagaagtgttgtgcctcggcccatcactcgtgggtctggatcctggtcttggcaaccccaggttgcgtccttgatgttccagagcttggtcttctgtgtggagaagagctcaccatctctacccaacttgagctttgggaccagactccctttagatcaaaccgccccatctgtggaagaactacaccagaagtcagcaagttttcagccaacagtgctggcctccccacctcccaggctgactagccctggggagaaggaaccctctcctcctagaccagcagagactccctgggcatgttcagtgtggccccacctcccttccagtcccagcttgcttcctccagctagcactaactcagcagcatcgctctgtggacgcctgtaaattattgagaaatgtgaactgtgcagtcttaaagctaaggtgttagaaaatttgatttatgctgtttagttgttgttgggtttcttttctttttaatttctttttcttttttgattttttttctttcccttaaaacaacagcagcagcatcttggctctttgtcatgtgttgaatggttgggtcttgtgaagtctgaggtctaacagtttattgtcctggaaggattttcttacagcagaaacagatttttttcaaattcccagaatcctgaggaccaagaaggatccctcagctgctacttccagcacccagcgtcactgggacgaaccaggccctgttcttacaaggccacatggctggccctttgcctccatggctactgtggtaagtgcagccttgtctgacccaatgctgacctaatgttggccattccacattgaggggacaaggtcagtgatgccccccttcactcacaagcacttcagaggcatgcagagagaagggacactcggccagctctctgaggtaatcagtgcaaggaggagtccgttttttgccagcaaacctcagcaggatcacactggaacagaacctggtcatacctgtgacaacacagctgtgagccagggcaaaccacccactgtcactggctcgagagtctgggcagaggctctgaccctccaccctttaaactggatgccggggcctggctgggcccaatgccaagtggttatggcaaccctgactatctggtcttaacatgtagctcaggaagtggaggcgctaatgtccccaatccctggggattcctgattccagctattcatgtaagcagagccaacctgcctatttctgtaggtgcgactgggatgttaggagcacagcaaggacccagctctgtagggctggtgacctgatacttctcataatggcatctagaagttaggctgagttggcctcactggcccagcaaaccagaacttgtctttgtccgggccatgttcttgggctgtcttctaattccaaagggttggttggtaaagctccacccccttctcctctgcctaaagacatcacatgtgtatacacacacgggtgtatagatgagttaaaagaatgtcctcgctggcatcctaattttgtcttaagtttttttggagggagaaaggaacaaggcaagggaagatgtgtagctttggctttaaccaggcagcctgggggctcccaagcctatggaaccctggtacaaagaagagaacagaagcgccctgtgaggagtgggatttgtttttctgtagaccagatgagaaggaaacaggccctgttttgtacatagttgcaacttaaaatttttggcttgcaaaatatttttgtaataaagatttctgggtaacaataaaaaaaaaaaaaaa

SEQ ID NO: 25 - protein, 172 aa, Mus musculus
MEPAGPAPGRLGPLLLCLLLSASCFCTDNNATHNWNVFIGVGVACALLVVLLMAALYLLRIKQKKAKGSTSSTRLHEPEKNAREITQIQDTNDINDITYADLNLPKEKKPAPRAPEPNNHTEYASIETGKVPRPEDTLTYADLDMVHLSRAQPAPKPEPSFSEYASVQVQRK

SEQ ID NO: 26 - DNA, 3393 bp, Mus musculus
actctaccctgcagccttcagcttggcacaaactaaacagtgactcttccccaagtgccgagtttaattcctggcttggccgaaaggattcagagagggataagcagcccctctggccttcagtgccaaaataagaaagagtatttcacatccacaagcaggaagtacacttcatacctctctaagataaaagacctattcacaatcaaaaatgtccctgcagatggtaacagtgggtcataacatagccttaattcaaccaggcttctcacttatgaattttgatggccaagttttcttctttggccagaaaggctggcctaagagatcctgtcctactggagtctttcattttgatataaaacaaaatcatctcaaactgaagcctgcaatcttctctaaagattcctgctacctcccacctcttcgttatccagctacttgctcatacaaaggcagcatagactctgacaagcatcaatatatcattcacggagggaaaacaccaaacaatgagctttccgataagatttatatcatgtctgtcgcttgcaagaataacaaaaaagttactttccgttgcacagagaaagacttagtaggagatgtccctgaacccagatacggccattccattgacgtggtgtatagtcgagggaaaagcatgggtgttctctttggaggacgttcatacatgccttctacccagagaaccacagaaaaatggaatagtgtagctgactgcctaccccatgttttcttgatagattttgaatttgggtgtgctacatcatatattctcccagaacttcaggatgggctgtcttttcatgtttctattgccagaaacgataccgtttatattttgggaggacactcacttgccagtaatatacgccctgctaacttgtatagaataagagtggaccttcccctgggtaccccagcagtgaattgcacagtcttgccaggaggaatctctgtctccagtgcaatcctcactcaaacaaacaatgatgaatttgttattgtgggtggttatcagctggaaaatcagaaaaggatggtctgcagccttgtctctctaggggacaacacgattgaaatcagtgagatggagactcctgactggacctcagatattaagcatagcaaaatatggtttggaagcaacatgggaaacgggactattttccttggcataccaggagacaataagcaggctatgtcagaagcattctatttctatactttgagatgctctgaagaggatttgagtgaagatcagaaaattgtctccaacagtcagacatcaacagaagatcctggggactccactccctttgaagactcagaggaattttgtttcagtgctgaagcaaccagttttgatggtgacgatgaatttgacacctacaatgaagatgatgaagatgacgagtctgtaaccggctactggataacatgttgccctacttgtgatgttgacatcaatacctgggttccgttctattcaacggagctcaataaacccgccatgatctattgttctcatggggatgggcactgggtacatgcccagtgcatggatttggaagaacgcacactcatccacttgtcagaaggaagcaacaagtattattgcaatgaacatgtacagatagcaagagcattgcaaactcccaaaagaaacccccccttacaaaaacctccaatgaaatccctccacaaaaaaggctctgggaaagtcttgactcctgccaagaaatccttccttagaagactgtttgattaatttagcaaaagcccctcagactcaggtatattgctctctgaatctactttcaatcataaacattattttgatttttgtttactgaaatctctatgttatgttttagttatgtgaattaagtgctgttgtgatttattgttaagtataactattctaatgtgtgttttttaacatcttatccaggaatgtcttaaatgagaaatgttatacagttttccattaaggatatcagtgataaagtatagaactcttacattattttgtaacaatctacatattgaatagtaactaaataccaataaataaactaatgcacaaaaagttaagttcttttgtgtaataagtagcctatagttggtttaaacagttaaaaccaacagctatatcccacactactgctgtttataaattttaaggtggcctctggtttatacttatgagcagaattatatatattggtcaataccatgaagaaaaatttaattctatatcaagccaggcatggtgatggtgatacatgcctgtaatcctggcacttaggaagtggaagaaggaagtttgtgagtttgatgcttgttgaggtatgaccttttgctatgtattgtagtgtatgagccccaagacctgcttgacccagagacaagagagtccacacatagatccaagtaatgctatgtgaccttgccccccggttacttgtgattaggtgaataaagatgtcaacagccaatagctgggcagaagagccaaaagtggggattgagggtaccctggcttgatgtaggaggagaccatgaggaaaggggagaaaaaagtgatggaggaggagaaagatgccatgagctaggagttaagaaagcatggccatgagtgctggccaattggagttaagagcagcccagatgaaacatagtaagtaataactcagggttatcgatagaaaatagattttagtgccgtactctccccagccctagagctgactatggcttactgtaaatataaagtttgtatgtgtcttttatccaggaactaaatggtcaaaggtggagtagaaactctggattgggattaaatttttctacaacaaatgctggcctgggctagattttatctcatatccgaaggctgacagaacacagagcactggtaacattgccacctgccatgcacaaagacctgagtctaatactgtggacattttcttgaagtatctacatgtacttctggagtgaaaacatattccaacaatatgcctttgtttaaatcactcactcactttgggccctcacattatatcctttcaaaatcaatggttcacccctttgaaaatgcttagccatagtccctcatcttccttaaagacagttgtcatctctggaaatagtcacatgtcattcaaggtccaatactgtgcagctctgaagtatggcattaccactttaagtgaaaagtgaaatatgaacatgagctcagacaaaggtttgggactatcactctcaaggaggctctactgctaagtcctgaactgctttcacatgaatacagaaattataacaaaaaatatgtaatcaataaaaagaaaactttcatattcc

SEQ ID NO: 27 - protein, 527 aa, Mus musculus
MSLQMVTVGHNIALIQPGFSLMNFDGQVFFFGQKGWPKRSCPTGVFHFDIKQNHLKLKPAIFSKDSCYLPPLRYPATCSYKGSIDSDKHQYIIHGGKTPNNELSDKIYIMSVACKNNKKVTFRCTEKDLVGDVPEPRYGHSIDVVYSRGKSMGVLFGGRSYMPSTQRTTEKWNSVADCLPHVFLIDFEFGCATSYILPELQDGLSFHVSIARNDTVYILGGHSLASNIRPANLYRIRVDLPLGTPAVNCTVLPGGISVSSAILTQTNNDEFVIVGGYQLENQKRMVCSLVSLGDNTIEISEMETPDWTSDIKHSKIWFGSNMGNGTIFLGIPGDNKQAMSEAFYFYTLRCSEEDLSEDQKIVSNSQTSTEDPGDSTPFEDSEEFCFSAEATSFDGDDEFDTYNEDDEDDESVTGYWITCCPTCDVDINTWVPFYSTELNKPAMIYCSHGDGHWVHAQCMDLEERTLIHLSEGSNKYYCNEHVQIARALQTPKRNPPLQKPPMKSLHKKGSGKVLTPAKKSFLRRLFD

SEQ ID NO: 28 - DNA, 1612 bp, Mus musculus
gacacagactacacccagagaaagaagagcaagcaccatgttgaaactattattgtcacctagatccttcttagtccttcagctgctcctgctgagggcagggtggagctccaaggtcctcatgtccagtgcgaatgaagacatcaaagctgatttgatcctgacttctacagcccctgaacacctcagtgctcctactctgccccttccagaggttcagtgctttgtgttcaacatagagtacatgaattgcacttggaatagcagttctgagcctcaggcaaccaacctcacgctgcactataggtacaaggtatctgataataatacattccaggagtgcagtcactatttgttctccaaagagattacttctggctgtcagatacaaaaagaagatatccagctctaccagacatttgttgtccagctccaggacccccagaaaccccagaggcgagctgtacagaagctaaacctacagaatcttgtgatcccacgggctccagaaaatctaacactcagcaatctgagtgaatcccagctagagctgagatggaaaagcagacatattaaagaacgctgtttacaatacttggtgcagtaccggagcaacagagatcgaagctggacggaactaatagtgaatcatgaacctagattctccctgcctagtgtggatgagctgaaacggtacacatttcgggttcggagccgctataacccaatctgtggaagttctcaacagtggagtaaatggagccagcctgtccactgggggagtcatactgtagaggagaatccttccttgtttgcactggaagctgtgcttatccctgttggcaccatggggttgattattaccctgatctttgtgtactgttggttggaacgaatgcctccaattccccccatcaagaatctagaggatctggttactgaataccaagggaacttttcggcctggagtggtgtgtctaaagggctgactgagagtctgcagccagactacagtgaacggttctgccacgtcagcgagattccccccaaaggaggggccctaggagaggggcctggaggttctccttgcagcctgcatagcccttactggcctcccccatgttattctctgaagccggaagcctgaacatcaatcctttgatggaacctcaaagtcctatagtcctaagtgacgctaacctcccctactcaccttggcaatctggatccaatgctcactgccttcccttggggctaagtttcgatttcctgtcccatgtaactgcttttctgttccatatgccctacttgagagtgtcccttgccctctttccctgcacaagccctcccatgcccagcctaacacctttccactttctttgaagagagtcttaccctgtagcccagggtggctgggagctcactatgtaggccaggttggcctccaactcacaggctatcctcccacctctgcctcataagagttggggttactggcatgcaccaccacacccagcatggtccttctcttttataggattctccctccctttttctacctatgattcaactgtttccaaatcaacaagaaataaagtttttaaccaatgat

SEQ ID NO: 29 - protein, 369 aa, Mus musculus
MLKLLLSPRSFLVLQLLLLRAGWSSKVLMSSANEDIKADLILTSTAPEHLSAPTLPLPEVQCFVFNIEYMNCTWNSSSEPQATNLTLHYRYKVSDNNTFQECSHYLFSKEITSGCQIQKEDIQLYQTFVVQLQDPQKPQRRAVQKLNLQNLVIPRAPENLTLSNLSESQLELRWKSRHIKERCLQYLVQYRSNRDRSWTELIVNHEPRFSLPSVDELKRYTFRVRSRYNPICGSSQQWSKWSQPVHWGSHTVEENPSLFALEAVLIPVGTMGLIITLIFVYCWLERMPPIPPIKNLEDLVTEYQGNFSAWSGVSKGLTESLQPDYSERFCHVSEIPPKGGALGEGPGGSPCSLHSPYWPPPCYSLKPEA

SEQ ID NO: 30 - DNA, 2012 bp, Homo sapiens
gttgggactccgggtggcaggcgcccgggggaatcccagctgactcgctcactgccttcgaagtccggcgccccccgggagggaactgggtggccgcaccctcccggctgcggtggctgtcgccccccaccctgcagccaggactcgatggagaatccattccaatatatggccatgtggctctttggagcaatgttccatcatgttccatgctgctgacgtcacatggagcacagaaatcaatgttagcagatagccagcccatacaagatcgtattgtattgtaggaggcattgtggatggatggctgctggaaaccccttgccatagccagctcttcttcaatacttaaggatttaccgtggctttgagtaatgagaatttcgaaaccacatttgagaagtatttccatccagtgctacttgtgtttacttctaaacagtcattttctaactgaagctggcattcatgtcttcattttgggctgtttcagtgcagggcttcctaaaacagaagccaactgggtgaatgtaataagtgatttgaaaaaaattgaagatcttattcaatctatgcatattgatgctactttatatacggaaagtgatgttcaccccagttgcaaagtaacagcaatgaagtgctttctcttggagttacaagttatttcacttgagtccggagatgcaagtattcatgatacagtagaaaatctgatcatcctagcaaacaacagtttgtcttctaatgggaatgtaacagaatctggatgcaaagaatgtgaggaactggaggaaaaaaatattaaagaatttttgcagagttttgtacatattgtccaaatgttcatcaacacttcttgattgcaattgattctttttaaagtgtttctgttattaacaaacatcactctgctgcttagacataacaaaacactcggcatttcaaatgtgctgtcaaaacaagtttttctgtcaagaagatgatcagaccttggatcagatgaactcttagaaatgaaggcagaaaaatgtcattgagtaatatagtgactatgaacttctctcagacttactttactcatttttttaatttattattgaaattgtacatatttgtggaataatgtaaaatgttgaataaaaatatgtacaagtgttgttttttaagttgcactgatattttacctcttattgcaaaatagcatttgtttaagggtgatagtcaaattatgtattggtggggctgggtaccaatgctgcaggtcaacagctatgctggtaggctcctgccagtgtggaaccactgactactggctctcattgacttccttactaagcatagcaaacagaggaagaatttgttatcagtaagaaaaagaagaactatatgtgaatcctcttctttatactgtaatttagttattgatgtataaagcaactgttatgaaataaagaaattgcaataactggcatataatgtccatcagtaaatcttggtggtggtggcaataataaacttctactgataggtagaatggtgtgcaagcttgtccaatcacggattgcaggccacatgcggcccaggacaactttgaatgtggcccaacacaaattcataaactttcatacatctcgtttttagctcatcagctatcattagcggtagtgtatttaaagtgtggcccaagacaattcttcttattccaatgtggcccagggaaatcaaaagattggatgcccctggtatagaaaactaatagtgacagtgttcatatttcatgctttcccaaatacaggtattttattttcacattctttttgccatgtttatataataataaagaaaaaccctgttgatttgttggagccattgttatctgacagaaaataattgtttatattttttgcactacactgtctaaaattagcaagctctcttctaatggaactgtaagaaagatgaaatatttttgttttattataaatttatttcaccttaaaaaaaaaaaa

SEQ ID NO: 31 - protein, 160 aa, Homo sapiens
MRISKPHLRSISIQCYLCLLLNSHFLTEAGIHVFILGCFSAGLPKTEANWVNVISDLKKIEDLIQSMHIDATLYTESDVHPSCKVTAMKCFLLELQVISLESGDASIHDTVENLIILANNSLSSNGNVTESGCKECEELEEKNIKEFLQSFVHIVQMFIN

SEQ ID NO: 32 - DNA, 2333 bp, Homo sapiens
gttgggactccgggtggcaggcgcccgggggaatcccagctgactcgctcactgccttcgaagtccggcgccccccgggagggaactgggtggccgcaccctcccggctgcggtggctgtcgccccccaccctgcagccaggactcgatggagaatccattccaatatatggccatgtggctctttggagcaatgttccatcatgttccatgctgctgacgtcacatggagcacagaaatcaatgttagcagatagccagcccatacaagatcgttttcaactagtggccccactgtgtccggaattgatgggttcttggtctcactgacttcaagaatgaagccgcggaccctcgcggtgagtgttacagctcttaaggtggcgcatctggagtttgttccttctgatgttcggatgtgttcggagtttcttccttctggtgggttcgtggtctcgctggctcaggagtgaagctacagaccttcgcggaggcattgtggatggatggctgctggaaaccccttgccatagccagctcttcttcaatacttaaggatttaccgtggctttgagtaatgagaatttcgaaaccacatttgagaagtatttccatccagtgctacttgtgtttacttctaaacagtcattttctaactgaagctggcattcatgtcttcattttgggatgcagctaatatacccagttggcccaaagcacctaacctatagttatataatctgactctcagttcagttttactctactaatgccttcatggtattgggaaccatagatttgtgcagctgtttcagtgcagggcttcctaaaacagaagccaactgggtgaatgtaataagtgatttgaaaaaaattgaagatcttattcaatctatgcatattgatgctactttatatacggaaagtgatgttcaccccagttgcaaagtaacagcaatgaagtgctttctcttggagttacaagttatttcacttgagtccggagatgcaagtattcatgatacagtagaaaatctgatcatcctagcaaacaacagtttgtcttctaatgggaatgtaacagaatctggatgcaaagaatgtgaggaactggaggaaaaaaatattaaagaatttttgcagagttttgtacatattgtccaaatgttcatcaacacttcttgattgcaattgattctttttaaagtgtttctgttattaacaaacatcactctgctgcttagacataacaaaacactcggcatttcaaatgtgctgtcaaaacaagtttttctgtcaagaagatgatcagaccttggatcagatgaactcttagaaatgaaggcagaaaaatgtcattgagtaatatagtgactatgaacttctctcagacttactttactcatttttttaatttattattgaaattgtacatatttgtggaataatgtaaaatgttgaataaaaatatgtacaagtgttgttttttaagttgcactgatattttacctcttattgcaaaatagcatttgtttaagggtgatagtcaaattatgtattggtggggctgggtaccaatgctgcaggtcaacagctatgctggtaggctcctgccagtgtggaaccactgactactggctctcattgacttccttactaagcatagcaaacagaggaagaatttgttatcagtaagaaaaagaagaactatatgtgaatcctcttctttatactgtaatttagttattgatgtataaagcaactgttatgaaataaagaaattgcaataactggcatataatgtccatcagtaaatcttggtggtggtggcaataataaacttctactgataggtagaatggtgtgcaagcttgtccaatcacggattgcaggccacatgcggcccaggacaactttgaatgtggcccaacacaaattcataaactttcatacatctcgtttttagctcatcagctatcattagcggtagtgtatttaaagtgtggcccaagacaattcttcttattccaatgtggcccagggaaatcaaaagattggatgcccctggtatagaaaactaatagtgacagtgttcatatttcatgctttcccaaatacaggtattttattttcacattctttttgccatgtttatataataataaagaaaaaccctgttgatttgttggagccattgttatctgacagaaaataattgtttatattttttgcactacactgtctaaaattagcaagctctcttctaatggaactgtaagaaagatgaaatatttttgttttattataaatttatttcaccttaaaaaaaaaaaa

SEQ ID NO: 33 - protein, 135 aa, Mus musculus
MVLGTIDLCSCFSAGLPKTEANWVNVISDLKKIEDLIQSMHIDATLYTESDVHPSCKVTAMKCFLLELQVISLESGDASIHDTVENLIILANNSLSSNGNVTESGCKECEELEEKNIKEFLQSFVHIVQMFINTS

SEQ ID NO: 34 - DNA, 1297 bp, Mus musculus
ttcttgaccaagacttcaatactcagtggcactgtattccccttctgtccagccactcttccccagagttctcttcttcatcctcccccttgcagagtagggcagcttgcaggtcctcctgcaagtctctcccaattctctgcgcccaaaagacttgcagtgcatctccttacgcgctgcagggaccttgccagggcaggactgcccccgcccagttgcagagttggacgaagacgggatcctgctgtgtttggaaggctgagttccacatctaacagctcagagaggtcaggaaagaatccaccttgacacatggccctctggctcttcaaagcactgcctcttcatggtccttgctggtgaggtccttaagaacacagaaacccatgtcagcagataaccagcctacaggaggccaagaagagttctggatggatggcagctggaagcccatcgccatagccagctcatcttcaacattgaagctcttacctgggcattaagtaatgaaaattttgaaaccatatatgaggaatacatccatctcgtgctacttgtgtttccttctaaacagtcactttttaactgaggctggcattcatgtcttcattttgggctgtgtcagtgtaggtctccctaaaacagaggccaactggatagatgtaagatatgacctggagaaaattgaaagccttattcaatctattcatattgacaccactttatacactgacagtgactttcatcccagttgcaaagttactgcaatgaactgctttctcctggaattgcaggttattttacatgagtacagtaacatgactcttaatgaaacagtaagaaacgtgctctaccttgcaaacagcactctgtcttctaacaagaatgtagcagaatctggctgcaaggaatgtgaggagctggaggagaaaaccttcacagagtttttgcaaagctttatacgcattgtccaaatgttcatcaacacgtcctgactgcatgcgagcctcttccgtgtttctgttattaaggtacctccacctgctgctcagaggcagcacagctccatgcatttgaaatctgctgggcaaactaagcttcctaacaaggagataatgagccacttggatcacatgaaatcttggaaatgaagagaggaaaagagctcgtctcagacttatttttgcttgcttatttttaatttattgcttcatttgtacatatttgtaatataacagaagatgtggaataaagttgtatggatattttatcaattgaaatttaaaaaaaaaaaaaa

SEQ ID NO: 35 - protein, 160 aa, Mus musculus
MKILKPYMRNTSISCYLCFLLNSHFLTEAGIHVFILGCVSVGLPKTEANWIDVRYDLEKIESLIQSIHIDTTLYTDSDFHPSCKVTAMNCFLLELQVILHEYSNMTLNETVRNVLYLANSTLSSNKNVAESGCKECEELEEKTFTEFLQSFIRIVQMFIN

SEQ ID NO: 36 - DNA, 1287 bp, Mus musculus
ttcttgaccaagacttcaatactcagtggcactgtattccccttctgtccagccactcttccccagagttctcttcttcatcctcccccttgcagagtagggcagcttgcaggtcctcctgcaagtctctcccaattctctgcgcccaaaagacttgcagtgcatctccttacgcgctgcagggaccttgccagggcaggactgcccccgcccagttgcagagttggacgaagacgggatcctgctgtgtttggaaggctgagttccacatctaacagctcagagagaatccaccttgacacatggccctctggctcttcaaagcactgcctcttcatggtccttgctggtgaggtccttaagaacacagaaacccatgtcagcagataaccagcctacaggaggccaagaagagttctggatggatggcagctggaagcccatcgccatagccagctcatcttcaacattgaagctcttacctgggcattaagtaatgaaaattttgaaaccatatatgaggaatacatccatctcgtgctacttgtgtttccttctaaacagtcactttttaactgaggctggcattcatgtcttcattttgggctgtgtcagtgtaggtctccctaaaacagaggccaactggatagatgtaagatatgacctggagaaaattgaaagccttattcaatctattcatattgacaccactttatacactgacagtgactttcatcccagttgcaaagttactgcaatgaactgctttctcctggaattgcaggttattttacatgagtacagtaacatgactcttaatgaaacagtaagaaacgtgctctaccttgcaaacagcactctgtcttctaacaagaatgtagcagaatctggctgcaaggaatgtgaggagctggaggagaaaaccttcacagagtttttgcaaagctttatacgcattgtccaaatgttcatcaacacgtcctgactgcatgcgagcctcttccgtgtttctgttattaaggtacctccacctgctgctcagaggcagcacagctccatgcatttgaaatctgctgggcaaactaagcttcctaacaaggagataatgagccacttggatcacatgaaatcttggaaatgaagagaggaaaagagctcgtctcagacttatttttgcttgcttatttttaatttattgcttcatttgtacatatttgtaatataacagaagatgtggaataaagttgtatggatattttatcaattgaaatttaaaaaaaaaaaaaa